European Patent Specification EP 4 081 666 B1, published August 21, 2024. Title: COMPOSITIONS AND METHODS FOR DETECTING METHICILLIN-RESISTANT STAPHYLOCOCCUS AUREUS. Applicant: F. Hoffmann-La Roche AG Roche Diagnostics GmbH Roche Molecular Systems, Inc. The sequence listing filed with the application follows.

SEQUENCE LISTING (7 sequences)

SEQ ID NO: 1 - DNA, 29 bp, Artificial Sequence
  mecA forward primer MECA_F1006
  modified_base (29)..(29): t-butyl-benzyl dC
atgatgcagttattggtaaaaagggactc

SEQ ID NO: 2 - DNA, 30 bp, Artificial Sequence
  mecA reverse primer MECA_R1077
  modified_base (30)..(30): t-butyl-benzyl dC
tgtatgtgcgattgtattgctattatcgtc

SEQ ID NO: 3 - DNA, 35 bp, Artificial Sequence
  mecA probe MECA_P2_TAO9
  misc_feature: 5` LCR_640 fluorophore
  misc_feature: 3` Iowa Black RQ blocker
  misc_feature (9)..(10): TAO quencher
ctccaacatgaagatggctatcgtgtcacaatcgt

SEQ ID NO: 4 - DNA, 29 bp, Artificial Sequence
  mecC forward primer MECC_F1_TBB
  modified_base (29)..(29): t-butyl-benzyl dA
acggcaatatcgatttaaagcaagcaata

SEQ ID NO: 5 - DNA, 22 bp, Artificial Sequence
  mecC forward primer MECC_F2_TBB
  modified_base (22)..(22): t-butyl-benzyl dA
tgcccgcattgcattagcatta

SEQ ID NO: 6 - DNA, 31 bp, Artificial Sequence
  mecC reverse primer MECC_R1_TBB
  modified_base (31)..(31): t-butyl-benzyl dA
tgctttataaaagggataatcactcgggata

SEQ ID NO: 7 - DNA, 33 bp, Artificial Sequence
  mecC probe MECCP1_LCR9.1
  misc_feature: 5` LCR 640 Fluorophore
  misc_feature: 3` Iowa Blacker RQ Blocker
  misc_feature (10)..(11): TAO Quencher
tgagcaaggtatgcaagatttgggaatcggtga